European Patent Specification EP 3 468 990 B1, published March 27, 2024. Title: Anti-C5 Antibodies and Uses Thereof. Applicant: Regeneron Pharmaceuticals, Inc. The sequence listing filed with the application follows.

SEQUENCE LISTING (366 sequences)

SEQ ID NO: 1 - DNA, 357 bp, Artificial Sequence
  synthetic
caggtgcagctggtggagtctgggggaggcgtggtccagcctggaaggtccctgagactctcctgtgtagcgtctggattcaccttcagtagttatggcattcactgggtccgccaggctccaggcaaggggctggagtgggtggcagttatatgggatgatggaaataatataaactattcagactccgtgaagggccgattcatcatctccagagacaattccaggaagacagtgtatctgcaaatgaacagcctgagaggcgaggacacggctgtttattactgtgcgagagatgcccccatagcaccagtccctgactattggggccagggaaccctggtcaccgtctcctca

SEQ ID NO: 2 - protein, 119 aa, Artificial Sequence
  synthetic
QVQLVESGGGVVQPGRSLRLSCVASGFTFSSYGIHWVRQAPGKGLEWVAVIWDDGNNINYSDSVKGRFIISRDNSRKTVYLQMNSLRGEDTAVYYCARDAPIAPVPDYWGQGTLVTVSS

SEQ ID NO: 3 - DNA, 24 bp, Artificial Sequence
  synthetic
ggattcaccttcagtagttatggc

SEQ ID NO: 4 - protein, 8 aa, Artificial Sequence
  synthetic
GFTFSSYG

SEQ ID NO: 5 - DNA, 24 bp, Artificial Sequence
  synthetic
atatgggatgatggaaataatata

SEQ ID NO: 6 - protein, 8 aa, Artificial Sequence
  synthetic
IWDDGNNI

SEQ ID NO: 7 - DNA, 36 bp, Artificial Sequence
  synthetic
gcgagagatgcccccatagcaccagtccctgactat

SEQ ID NO: 8 - protein, 12 aa, Artificial Sequence
  synthetic
ARDAPIAPVPDY

SEQ ID NO: 9 - DNA, 321 bp, Artificial Sequence
  synthetic
gacatccagatgacccagtctccttccaccctgtctgcatctgtaggagacagagtcaccatcacttgccgggccagtcagagtattagtagttggttggcctggtatcagcagaaaccagggaaagcccctaagctcctgatctataaggcgtctagtttagacactggggtcccatcaaggttcagcggcagtggatctgggacagagttcactctcaccatcagcagcctgcagcctgatgattttgcaacttattactgccaacagtataatacttattcgtacacttttggcctggggaccaaactggagatcaaa

SEQ ID NO: 10 - protein, 107 aa, Artificial Sequence
  synthetic
DIQMTQSPSTLSASVGDRVTITCRASQSISSWLAWYQQKPGKAPKLLIYKASSLDTGVPSRFSGSGSGTEFTLTISSLQPDDFATYYCQQYNTYSYTFGLGTKLEIK

SEQ ID NO: 11 - DNA, 18 bp, Artificial Sequence
  synthetic
cagagtattagtagttgg

SEQ ID NO: 12 - protein, 6 aa, Artificial Sequence
  synthetic
QSISSW

SEQ ID NO: 13 - DNA, 9 bp, Artificial Sequence
  synthetic
aaggcgtct

SEQ ID NO: 14 - protein, 3 aa, Artificial Sequence
  synthetic
KAS

SEQ ID NO: 15 - DNA, 27 bp, Artificial Sequence
  synthetic
caacagtataatacttattcgtacact

SEQ ID NO: 16 - protein, 9 aa, Artificial Sequence
  synthetic
QQYNTYSYT

SEQ ID NO: 17 - DNA, 357 bp, Artificial Sequence
  synthetic
caggtgcaactggtggagtctgggggaggcttggtcaagcctggagggtccctgagactctcctgtgcagcttctggattcaccttcagtgactactacatgagctggatccgccaggctccagggaaggggctggagtgggtttcatatattagcagtagtggtaataccataaaatatgcagactctatgaagggccgattcaccatctccagggacaacgccaagaaatcactgtttgtggaaatgaacagcctgagagccgaggacacggccgtgtattactgtgcgaggtataaaagttcgtccgactactttgaccactggggccagggaaccctggtcaccgtctcctca

SEQ ID NO: 18 - protein, 119 aa, Artificial Sequence
  synthetic
QVQLVESGGGLVKPGGSLRLSCAASGFTFSDYYMSWIRQAPGKGLEWVSYISSSGNTIKYADSMKGRFTISRDNAKKSLFVEMNSLRAEDTAVYYCARYKSSSDYFDHWGQGTLVTVSS

SEQ ID NO: 19 - DNA, 24 bp, Artificial Sequence
  synthetic
ggattcaccttcagtgactactac

SEQ ID NO: 20 - protein, 8 aa, Artificial Sequence
  synthetic
GFTFSDYY

SEQ ID NO: 21 - DNA, 24 bp, Artificial Sequence
  synthetic
attagcagtagtggtaataccata

SEQ ID NO: 22 - protein, 8 aa, Artificial Sequence
  synthetic
ISSSGNTI

SEQ ID NO: 23 - DNA, 36 bp, Artificial Sequence
  synthetic
gcgaggtataaaagttcgtccgactactttgaccac

SEQ ID NO: 24 - protein, 12 aa, Artificial Sequence
  synthetic
ARYKSSSDYFDH

SEQ ID NO: 25 - DNA, 321 bp, Artificial Sequence
  synthetic
gaaattgtgttgacacagtctccagccaccctgtctttgtctccaggggaaagagccaccctctcctgcagggccagtcagagtgttaggagttacttagcctggtaccaacagaaacctggccaggctcccaggctcctcatctatgatgcatccaacagggccactgccatcccagccaggttcagtggcagtgggtctgggacagacttcactctcaccatcagcagcctagagcctgaagatttagcagtttattactgtcagcagtctggcaactggccgctcactttcggcggagggaccaaggtggagatcaaa

SEQ ID NO: 26 - protein, 107 aa, Artificial Sequence
  synthetic
EIVLTQSPATLSLSPGERATLSCRASQSVRSYLAWYQQKPGQAPRLLIYDASNRATAIPARFSGSGSGTDFTLTISSLEPEDLAVYYCQQSGNWPLTFGGGTKVEIK

SEQ ID NO: 27 - DNA, 18 bp, Artificial Sequence
  synthetic
cagagtgttaggagttac

SEQ ID NO: 28 - protein, 6 aa, Artificial Sequence
  synthetic
QSVRSY

SEQ ID NO: 29 - DNA, 9 bp, Artificial Sequence
  synthetic
gatgcatcc

SEQ ID NO: 30 - protein, 3 aa, Artificial Sequence
  synthetic
DAS

SEQ ID NO: 31 - DNA, 27 bp, Artificial Sequence
  synthetic
cagcagtctggcaactggccgctcact

SEQ ID NO: 32 - protein, 9 aa, Artificial Sequence
  synthetic
QQSGNWPLT

SEQ ID NO: 33 - DNA, 357 bp, Artificial Sequence
  synthetic
caggtgcagctggtggagtctgggggaggcgtggtccagcctgggaggtccttgagactctcctgtggagcgtctggattcaccttcagtacttatggcatgcactgggtccgccaggctccaggcaaggggctggagtgggtggcagttatctgggatgatggaaataataaatattatgcagactccgtgaagggccgattcaccatctccagagacaattcgaagaacacgctgtatctgcagatgaacagcctgagagccgaggacacggctgtttattactgtgcgagagattcagaggtcgccccagttggggactactggggccagggcaccctggtcaccgtctcctca

SEQ ID NO: 34 - protein, 119 aa, Artificial Sequence
  synthetic
QVQLVESGGGVVQPGRSLRLSCGASGFTFSTYGMHWVRQAPGKGLEWVAVIWDDGNNKYYADSVKGRFTISRDNSKNTLYLQMNSLRAEDTAVYYCARDSEVAPVGDYWGQGTLVTVSS

SEQ ID NO: 35 - DNA, 24 bp, Artificial Sequence
  synthetic
ggattcaccttcagtacttatggc

SEQ ID NO: 36 - protein, 8 aa, Artificial Sequence
  synthetic
GFTFSTYG

SEQ ID NO: 37 - DNA, 24 bp, Artificial Sequence
  synthetic
atctgggatgatggaaataataaa

SEQ ID NO: 38 - protein, 8 aa, Artificial Sequence
  synthetic
IWDDGNNK

SEQ ID NO: 39 - DNA, 36 bp, Artificial Sequence
  synthetic
gcgagagattcagaggtcgccccagttggggactac

SEQ ID NO: 40 - protein, 12 aa, Artificial Sequence
  synthetic
ARDSEVAPVGDY

SEQ ID NO: 41 - DNA, 321 bp, Artificial Sequence
  synthetic
gacatccagatgacccagtctccttccaccctgtctgcatctgtaggagacagagtcactatcatttgccgggccagtcagagtattaacaggtggttggcctggtatcagcagaaaccagggaaggcccctaaactcctgatctataaggcgtctagtttagaaagtggggtcccatcaaggttcagcggcagtggatctgggacagaattcactctcaccatcagcagcctgcagcctgatgattttgcagcttattactgccaacagtataatgattattcgtacacttttggccaggggaccaagctggagatcaaa

SEQ ID NO: 42 - protein, 107 aa, Artificial Sequence
  synthetic
DIQMTQSPSTLSASVGDRVTIICRASQSINRWLAWYQQKPGKAPKLLIYKASSLESGVPSRFSGSGSGTEFTLTISSLQPDDFAAYYCQQYNDYSYTFGQGTKLEIK

SEQ ID NO: 43 - DNA, 18 bp, Artificial Sequence
  synthetic
cagagtattaacaggtgg

SEQ ID NO: 44 - protein, 6 aa, Artificial Sequence
  synthetic
QSINRW

SEQ ID NO: 45 - DNA, 9 bp, Artificial Sequence
  synthetic
aaggcgtct

SEQ ID NO: 46 - protein, 3 aa, Artificial Sequence
  synthetic
KAS

SEQ ID NO: 47 - DNA, 27 bp, Artificial Sequence
  synthetic
caacagtataatgattattcgtacact

SEQ ID NO: 48 - protein, 9 aa, Artificial Sequence
  synthetic
QQYNDYSYT

SEQ ID NO: 49 - DNA, 366 bp, Artificial Sequence
  synthetic
gaggtgcagctggtggagtctgggggagacttggtccagcctggagggtccctgagactctcctgtgcagcctctggattcaccttcagtgaccactatatggactgggtccgccaggctccagggaaggggctggactggattggccgtattagaaacaaagctaacgcttataacacagaatacgccgcgtctgtgagaggcagattcaccatctcaagagatgattcacagaatttactgtatctgcaaatgaacagcctgaaaaccgatgacacggccgtatattattgtgttagagtctggaactacgcctacttcgctatggacgtctggggccaagggaccacggtcaccgtctcctca

SEQ ID NO: 50 - protein, 122 aa, Artificial Sequence
  synthetic
EVQLVESGGDLVQPGGSLRLSCAASGFTFSDHYMDWVRQAPGKGLDWIGRIRNKANAYNTEYAASVRGRFTISRDDSQNLLYLQMNSLKTDDTAVYYCVRVWNYAYFAMDVWGQGTTVTVSS

SEQ ID NO: 51 - DNA, 24 bp, Artificial Sequence
  synthetic
ggattcaccttcagtgaccactat

SEQ ID NO: 52 - protein, 8 aa, Artificial Sequence
  synthetic
GFTFSDHY

SEQ ID NO: 53 - DNA, 30 bp, Artificial Sequence
  synthetic
attagaaacaaagctaacgcttataacaca

SEQ ID NO: 54 - protein, 10 aa, Artificial Sequence
  synthetic
IRNKANAYNT

SEQ ID NO: 55 - DNA, 39 bp, Artificial Sequence
  synthetic
gttagagtctggaactacgcctacttcgctatggacgtc

SEQ ID NO: 56 - protein, 13 aa, Artificial Sequence
  synthetic
VRVWNYAYFAMDV

SEQ ID NO: 57 - DNA, 321 bp, Artificial Sequence
  synthetic
gacatccagatgacccagtctccatcctccctatctgcatctgtgggagacagagtcaccatcacttgccggtcaagtcagaacattggaatctttttaaactggtatcaacaaaaaccaggggaagcccctaacctcctgatctccgctgcatccagtttacacagtggggtcccttcaaggttcagtggcagtgggtctgggacagatttcactctcaccatcggcagtctgcagcctgaagattttgcgacttactactgtcaacagacgtacaataccatattcactttcggccctgggaccaaagtggatatcaaa

SEQ ID NO: 58 - protein, 107 aa, Artificial Sequence
  synthetic
DIQMTQSPSSLSASVGDRVTITCRSSQNIGIFLNWYQQKPGEAPNLLISAASSLHSGVPSRFSGSGSGTDFTLTIGSLQPEDFATYYCQQTYNTIFTFGPGTKVDIK

SEQ ID NO: 59 - DNA, 18 bp, Artificial Sequence
  synthetic
cagaacattggaatcttt

SEQ ID NO: 60 - protein, 6 aa, Artificial Sequence
  synthetic
QNIGIF

SEQ ID NO: 61 - DNA, 9 bp, Artificial Sequence
  synthetic
gctgcatcc

SEQ ID NO: 62 - protein, 3 aa, Artificial Sequence
  synthetic
AAS

SEQ ID NO: 63 - DNA, 27 bp, Artificial Sequence
  synthetic
caacagacgtacaataccatattcact

SEQ ID NO: 64 - protein, 9 aa, Artificial Sequence
  synthetic
QQTYNTIFT

SEQ ID NO: 65 - DNA, 363 bp, Artificial Sequence
  synthetic
gaggtgcagctggtggagtctgggggagacttggtacagcctggggggtccctgagactctcctgtgcagcctctggattcacctttagcagctatgccatgaactgggtccgccagggtccagggaagggactggagtgggtctcagctattagtggtcgtggtgatagtacatactacgcagactccgtgaagggccggctcaccatctccagagacaattccaagaacacgctgtatctgcaaatgaacagcctgagagccgaggacacggccgtatattactgtgtgaaagagggggagcaactcgtctactggtacttcgatctctggggccgtggcaccctggtcaccgtctcctca

SEQ ID NO: 66 - protein, 121 aa, Artificial Sequence
  synthetic
EVQLVESGGDLVQPGGSLRLSCAASGFTFSSYAMNWVRQGPGKGLEWVSAISGRGDSTYYADSVKGRLTISRDNSKNTLYLQMNSLRAEDTAVYYCVKEGEQLVYWYFDLWGRGTLVTVSS

SEQ ID NO: 67 - DNA, 24 bp, Artificial Sequence
  synthetic
ggattcacctttagcagctatgcc

SEQ ID NO: 68 - protein, 8 aa, Artificial Sequence
  synthetic
GFTFSSYA

SEQ ID NO: 69 - DNA, 24 bp, Artificial Sequence
  synthetic
attagtggtcgtggtgatagtaca

SEQ ID NO: 70 - protein, 8 aa, Artificial Sequence
  synthetic
ISGRGDST

SEQ ID NO: 71 - DNA, 42 bp, Artificial Sequence
  synthetic
gtgaaagagggggagcaactcgtctactggtacttcgatctc

SEQ ID NO: 72 - protein, 14 aa, Artificial Sequence
  synthetic
VKEGEQLVYWYFDL

SEQ ID NO: 73 - DNA, 321 bp, Artificial Sequence
  synthetic
gacatccagatgacccagtctccatcctccctgtctgcatctgtaggagacagagtcaccatcacttgccgggcaagtcagaccattagcaactttttacattggtatcagcagaaaccagggaaagcccctaagctcctgatctatgctgcatccagtttgcaaagtggggtcccatcaaggttcagtggcagtggatctgggacagatttcactctcaccatcagcagtctgcaacctgaagatttttcaacttacttctgtcaacagagttacactaccccgctcactttcggcggagggaccaaggtggagatcaaa

SEQ ID NO: 74 - protein, 107 aa, Artificial Sequence
  synthetic
DIQMTQSPSSLSASVGDRVTITCRASQTISNFLHWYQQKPGKAPKLLIYAASSLQSGVPSRFSGSGSGTDFTLTISSLQPEDFSTYFCQQSYTTPLTFGGGTKVEIK

SEQ ID NO: 75 - DNA, 18 bp, Artificial Sequence
  synthetic
cagaccattagcaacttt

SEQ ID NO: 76 - protein, 6 aa, Artificial Sequence
  synthetic
QTISNF

SEQ ID NO: 77 - DNA, 9 bp, Artificial Sequence
  synthetic
gctgcatcc

SEQ ID NO: 78 - protein, 3 aa, Artificial Sequence
  synthetic
AAS

SEQ ID NO: 79 - DNA, 27 bp, Artificial Sequence
  synthetic
caacagagttacactaccccgctcact

SEQ ID NO: 80 - protein, 9 aa, Artificial Sequence
  synthetic
QQSYTTPLT

SEQ ID NO: 81 - DNA, 363 bp, Artificial Sequence
  synthetic
gaggtgcagctggtggagtctgggggaggcttggtgaggtcgggggggtccctgagactctcctgtgcagcctctggattcacctttaacagatatgccatgacctgggtccgccaggctccagggaaggggctggagtgggtctcagctataagtggtagtggtagcagcacatactacacagactccgtgaaaggccggttcaccatctccagagacaattccaagaattcggtggatctgcaaatgcacagcctgagagtcgaagacacggccatatattattgtgcgagagggactacagtcactacggggtacggtatggacgtctggggccaagggaccacggtcaccgtctcctca

SEQ ID NO: 82 - protein, 121 aa, Artificial Sequence
  synthetic
EVQLVESGGGLVRSGGSLRLSCAASGFTFNRYAMTWVRQAPGKGLEWVSAISGSGSSTYYTDSVKGRFTISRDNSKNSVDLQMHSLRVEDTAIYYCARGTTVTTGYGMDVWGQGTTVTVSS

SEQ ID NO: 83 - DNA, 24 bp, Artificial Sequence
  synthetic
ggattcacctttaacagatatgcc

SEQ ID NO: 84 - protein, 8 aa, Artificial Sequence
  synthetic
GFTFNRYA

SEQ ID NO: 85 - DNA, 24 bp, Artificial Sequence
  synthetic
ataagtggtagtggtagcagcaca

SEQ ID NO: 86 - protein, 8 aa, Artificial Sequence
  synthetic
ISGSGSST

SEQ ID NO: 87 - DNA, 42 bp, Artificial Sequence
  synthetic
gcgagagggactacagtcactacggggtacggtatggacgtc

SEQ ID NO: 88 - protein, 14 aa, Artificial Sequence
  synthetic
ARGTTVTTGYGMDV

SEQ ID NO: 89 - DNA, 321 bp, Artificial Sequence
  synthetic
gacatccagatgacccagtctccatcctccctgtctgcatctgtaggagacagagtcaccttcacttgccaggcgagtcaggacattaccaattctttaaattggtatcaacagaaacctgggagagcccctaagctcctgatctacgatgcatcgtatttgaaggcaggggtcccatcaagattcagtggaagtggatctgggacagattttactttcaccatcagcagcctgcagcctgaagatattgcaacatattactgtcaacaatatgatgatctcccatacacttttggccaggggaccaagctggagatcaaa

SEQ ID NO: 90 - protein, 107 aa, Artificial Sequence
  synthetic
DIQMTQSPSSLSASVGDRVTFTCQASQDITNSLNWYQQKPGRAPKLLIYDASYLKAGVPSRFSGSGSGTDFTFTISSLQPEDIATYYCQQYDDLPYTFGQGTKLEIK

SEQ ID NO: 91 - DNA, 18 bp, Artificial Sequence
  synthetic
caggacattaccaattct

SEQ ID NO: 92 - protein, 6 aa, Artificial Sequence
  synthetic
QDITNS

SEQ ID NO: 93 - DNA, 9 bp, Artificial Sequence
  synthetic
gatgcatcg

SEQ ID NO: 94 - protein, 3 aa, Artificial Sequence
  synthetic
DAS

SEQ ID NO: 95 - DNA, 27 bp, Artificial Sequence
  synthetic
caacaatatgatgatctcccatacact

SEQ ID NO: 96 - protein, 9 aa, Artificial Sequence
  synthetic
QQYDDLPYT

SEQ ID NO: 97 - DNA, 360 bp, Artificial Sequence
  synthetic
caggtgcagctgcaggagtcgggcccaggactggtgaagccttcggagaccctgtccctcacctgcactgtctctggtgactccgtcagtagttcctactggacctggatccggcagcccccagggaagggactggagtggattggctatatctattacagtgggagttccaactacaacccctccctcaagagtcgagccaccatttcagtagacacgtccaagaaccagttctccctgaagctgagttctgtgaccgctgcggacacggccgtatattactgtgcgagagaagggaacgtggatacaactatgatatttgactactggggccagggaaccctggtcaccgtctcctca

SEQ ID NO: 98 - protein, 120 aa, Artificial Sequence
  synthetic
QVQLQESGPGLVKPSETLSLTCTVSGDSVSSSYWTWIRQPPGKGLEWIGYIYYSGSSNYNPSLKSRATISVDTSKNQFSLKLSSVTAADTAVYYCAREGNVDTTMIFDYWGQGTLVTVSS

SEQ ID NO: 99 - DNA, 24 bp, Artificial Sequence
  synthetic
ggtgactccgtcagtagttcctac

SEQ ID NO: 100 - protein, 8 aa, Artificial Sequence
  synthetic
GDSVSSSY

SEQ ID NO: 101 - DNA, 21 bp, Artificial Sequence
  synthetic
atctattacagtgggagttcc

SEQ ID NO: 102 - protein, 7 aa, Artificial Sequence
  synthetic
IYYSGSS

SEQ ID NO: 103 - DNA, 42 bp, Artificial Sequence
  synthetic
gcgagagaagggaacgtggatacaactatgatatttgactac

SEQ ID NO: 104 - protein, 14 aa, Artificial Sequence
  synthetic
AREGNVDTTMIFDY

SEQ ID NO: 105 - DNA, 321 bp, Artificial Sequence
  synthetic
gccatccagatgacccagtctccatcctccctgtctgcatctgtaggagacagagtcaccatcacttgccgggcaagtcagggcattagaaatgatttaggctggtatcaacagaaaccagggaaagcccctaaactcctgatctatgctgcatccagtttacaaagtggggtcccatcgaggttcgccggccgtggatctggcacagatttcactctcaccatcagcagcctgcagcctgaagattttgcaacttattactgtctacaagatttcaattacccgtggacgttcggccaagggaccaaggtggaaatcaaa

SEQ ID NO: 106 - protein, 107 aa, Artificial Sequence
  synthetic
AIQMTQSPSSLSASVGDRVTITCRASQGIRNDLGWYQQKPGKAPKLLIYAASSLQSGVPSRFAGRGSGTDFTLTISSLQPEDFATYYCLQDFNYPWTFGQGTKVEIK

SEQ ID NO: 107 - DNA, 18 bp, Artificial Sequence
  synthetic
cagggcattagaaatgat

SEQ ID NO: 108 - protein, 6 aa, Artificial Sequence
  synthetic
QGIRND

SEQ ID NO: 109 - DNA, 9 bp, Artificial Sequence
  synthetic
gctgcatcc

SEQ ID NO: 110 - protein, 3 aa, Artificial Sequence
  synthetic
AAS

SEQ ID NO: 111 - DNA, 27 bp, Artificial Sequence
  synthetic
ctacaagatttcaattacccgtggacg

SEQ ID NO: 112 - protein, 9 aa, Artificial Sequence
  synthetic
LQDFNYPWT

SEQ ID NO: 113 - DNA, 321 bp, Artificial Sequence
  synthetic
gccatccagatgacccagtctccatcctccctgtctgcatctgtaggagacagagtcaccatcacttgccgggcaagtcagggcattagaaatgatttaggctggtatcaacagaaaccagggaaagcccctaaactcctgatctatgctgcatccagtttacaaagtggggtcccatcgaggttcgccggccgtggatctggcacagatttcactctcaccatcagcagcctgcagcctgaagattttgcaacttattactgtcatcaagatttcaattacccgtggacgttcggccaagggaccaaggtggaaatcaaa

SEQ ID NO: 114 - protein, 107 aa, Artificial Sequence
  synthetic
AIQMTQSPSSLSASVGDRVTITCRASQGIRNDLGWYQQKPGKAPKLLIYAASSLQSGVPSRFAGRGSGTDFTLTISSLQPEDFATYYCHQDFNYPWTFGQGTKVEIK

SEQ ID NO: 115 - DNA, 18 bp, Artificial Sequence
  synthetic
cagggcattagaaatgat

SEQ ID NO: 116 - protein, 6 aa, Artificial Sequence
  synthetic
QGIRND

SEQ ID NO: 117 - DNA, 9 bp, Artificial Sequence
  synthetic
gctgcatcc

SEQ ID NO: 118 - protein, 3 aa, Artificial Sequence
  synthetic
AAS

SEQ ID NO: 119 - DNA, 27 bp, Artificial Sequence
  synthetic
catcaagatttcaattacccgtggacg

SEQ ID NO: 120 - protein, 9 aa, Artificial Sequence
  synthetic
HQDFNYPWT

SEQ ID NO: 121 - DNA, 360 bp, Artificial Sequence
  synthetic
caggtgcagctgcaggagtcgggcccaggactggtgaagccttcggagaccctgtccctcacctgcactgtctctggtgactccgtcagtagttcctactggacctggatccggcagcccccagggaagggactggagtggattggctatatctattacagtgggagttccaactacaacccctccctcaagagtcgagccaccatttcagtagacacgtccaagaaccagttctccctgaagctgagttctgtgaccgctgcggacacggccgtatattactgtgcgagagaacataacgtggatacaactatgatatttgactactggggccagggaaccctggtcaccgtctcctca

SEQ ID NO: 122 - protein, 120 aa, Artificial Sequence
  synthetic
QVQLQESGPGLVKPSETLSLTCTVSGDSVSSSYWTWIRQPPGKGLEWIGYIYYSGSSNYNPSLKSRATISVDTSKNQFSLKLSSVTAADTAVYYCAREHNVDTTMIFDYWGQGTLVTVSS

SEQ ID NO: 123 - DNA, 24 bp, Artificial Sequence
  synthetic
ggtgactccgtcagtagttcctac

SEQ ID NO: 124 - protein, 8 aa, Artificial Sequence
  synthetic
GDSVSSSY

SEQ ID NO: 125 - DNA, 21 bp, Artificial Sequence
  synthetic
atctattacagtgggagttcc

SEQ ID NO: 126 - protein, 7 aa, Artificial Sequence
  synthetic
IYYSGSS

SEQ ID NO: 127 - DNA, 42 bp, Artificial Sequence
  synthetic
gcgagagaacataacgtggatacaactatgatatttgactac

SEQ ID NO: 128 - protein, 14 aa, Artificial Sequence
  synthetic
AREHNVDTTMIFDY

SEQ ID NO: 129 - DNA, 321 bp, Artificial Sequence
  synthetic
gccatccagatgacccagtctccatcctccctgtctgcatctgtaggagacagagtcaccatcacttgccgggcaagtcagggcattagaaatgatttaggctggtatcaacagaaaccagggaaagcccctaaactcctgatctatgctgcatccagtttacaaagtggggtcccatcgaggttcgccggccgtggatctggcacagatttcactctcaccatcagcagcctgcagcctgaagattttgcaacttattactgtctacaagatttcaattacccgtggcacttcggccaagggaccaaggtggaaatcaaa

SEQ ID NO: 130 - protein, 107 aa, Artificial Sequence
  synthetic
AIQMTQSPSSLSASVGDRVTITCRASQGIRNDLGWYQQKPGKAPKLLIYAASSLQSGVPSRFAGRGSGTDFTLTISSLQPEDFATYYCLQDFNYPWHFGQGTKVEIK

SEQ ID NO: 131 - DNA, 18 bp, Artificial Sequence
  synthetic
cagggcattagaaatgat

SEQ ID NO: 132 - protein, 6 aa, Artificial Sequence
  synthetic
QGIRND

SEQ ID NO: 133 - DNA, 9 bp, Artificial Sequence
  synthetic
gctgcatcc

SEQ ID NO: 134 - protein, 3 aa, Artificial Sequence
  synthetic
AAS

SEQ ID NO: 135 - DNA, 27 bp, Artificial Sequence
  synthetic
ctacaagatttcaattacccgtggcac

SEQ ID NO: 136 - protein, 9 aa, Artificial Sequence
  synthetic
LQDFNYPWH

SEQ ID NO: 137 - DNA, 360 bp, Artificial Sequence
  synthetic
caggtgcagctgcaggagtcgggcccaggactggtgaagccttcggagaccctgtccctcacctgcactgtctctggtgactccgtcagtagttcctactggacctggatccggcagcccccagggaagggactggagtggattggctatatctattacagtgggagttccaactacaacccctccctcaagagtcgagccaccatttcagtagacacgtccaagaaccagttctccctgaagctgagttctgtgaccgctgcggacacggccgtatattactgtgcgagagaagggaacgtggatacaactatgatacatgactactggggccagggaaccctggtcaccgtctcctca

SEQ ID NO: 138 - protein, 120 aa, Artificial Sequence
  synthetic
QVQLQESGPGLVKPSETLSLTCTVSGDSVSSSYWTWIRQPPGKGLEWIGYIYYSGSSNYNPSLKSRATISVDTSKNQFSLKLSSVTAADTAVYYCAREGNVDTTMIHDYWGQGTLVTVSS

SEQ ID NO: 139 - DNA, 24 bp, Artificial Sequence
  synthetic
ggtgactccgtcagtagttcctac

SEQ ID NO: 140 - protein, 8 aa, Artificial Sequence
  synthetic
GDSVSSSY

SEQ ID NO: 141 - DNA, 21 bp, Artificial Sequence
  synthetic
atctattacagtgggagttcc

SEQ ID NO: 142 - protein, 7 aa, Artificial Sequence
  synthetic
IYYSGSS

SEQ ID NO: 143 - DNA, 42 bp, Artificial Sequence
  synthetic
gcgagagaagggaacgtggatacaactatgatacatgactac

SEQ ID NO: 144 - protein, 14 aa, Artificial Sequence
  synthetic
AREGNVDTTMIHDY

SEQ ID NO: 145 - DNA, 360 bp, Artificial Sequence
  synthetic
caggtgcagctgcaggagtcgggcccaggactggtgaagccttcggagaccctgtccctcacctgcactgtctctggtgactccgtcagtagttcctactggacctggatccggcagcccccagggaagggactggagtggattggctatatctattacagtgggagttccaactacaacccctccctcaagagtcgagccaccatttcagtagacacgtccaagaaccagttctccctgaagctgagttctgtgaccgctgcggacacggccgtatattactgtgcgagagaagggaacgtggatcacactatgatatttgactactggggccagggaaccctggtcaccgtctcctca

SEQ ID NO: 146 - protein, 120 aa, Artificial Sequence
  synthetic
QVQLQESGPGLVKPSETLSLTCTVSGDSVSSSYWTWIRQPPGKGLEWIGYIYYSGSSNYNPSLKSRATISVDTSKNQFSLKLSSVTAADTAVYYCAREGNVDHTMIFDYWGQGTLVTVSS

SEQ ID NO: 147 - DNA, 24 bp, Artificial Sequence
  synthetic
ggtgactccgtcagtagttcctac

SEQ ID NO: 148 - protein, 8 aa, Artificial Sequence
  synthetic
GDSVSSSY

SEQ ID NO: 149 - DNA, 21 bp, Artificial Sequence
  synthetic
atctattacagtgggagttcc

SEQ ID NO: 150 - protein, 7 aa, Artificial Sequence
  synthetic
IYYSGSS

SEQ ID NO: 151 - DNA, 42 bp, Artificial Sequence
  synthetic
gcgagagaagggaacgtggatcacactatgatatttgactac

SEQ ID NO: 152 - protein, 14 aa, Artificial Sequence
  synthetic
AREGNVDHTMIFDY

SEQ ID NO: 153 - DNA, 360 bp, Artificial Sequence
  synthetic
caggtgcagctggtggagtctgggggaggcttggtcaagcctggagggtccctgagactctcctgtgcagcctctggattcaccttcagtgactcctacatgtcctggatccgtcaggctccagggaagggactagagtggatttcatacattggtagtagtggtaataccttttactacgcagactctgtgaagggccggttcaccatttccagagacaacgccaacaatttactgtatctgcaaatgaccagcctgagagccgaggacacggccgtgtattactgtgcgagagaagaaggcgatttttggagtgccgttgactcctggggccagggaaccctggtcaccgtctcctca

SEQ ID NO: 154 - protein, 120 aa, Artificial Sequence
  synthetic
QVQLVESGGGLVKPGGSLRLSCAASGFTFSDSYMSWIRQAPGKGLEWISYIGSSGNTFYYADSVKGRFTISRDNANNLLYLQMTSLRAEDTAVYYCAREEGDFWSAVDSWGQGTLVTVSS

SEQ ID NO: 155 - DNA, 24 bp, Artificial Sequence
  synthetic
ggattcaccttcagtgactcctac

SEQ ID NO: 156 - protein, 8 aa, Artificial Sequence
  synthetic
GFTFSDSY

SEQ ID NO: 157 - DNA, 24 bp, Artificial Sequence
  synthetic
attggtagtagtggtaataccttt

SEQ ID NO: 158 - protein, 8 aa, Artificial Sequence
  synthetic
IGSSGNTF

SEQ ID NO: 159 - DNA, 39 bp, Artificial Sequence
  synthetic
gcgagagaagaaggcgatttttggagtgccgttgactcc

SEQ ID NO: 160 - protein, 13 aa, Artificial Sequence
  synthetic
AREEGDFWSAVDS

SEQ ID NO: 161 - DNA, 321 bp, Artificial Sequence
  synthetic
gacatccagttgacccagtctccatccttcctgtctgcatctgtaggagacagagtcaccatcacttgctgggccagtcagggcattagcagttatttagcctggtatcagcaaaaaccaggtaaagcccctaaactcctgatccatactgcatccactttgcaaagtggggtcccatcaaggttcagcggcagtggatctgggacagaattcactctcacaatcagcaacctgcagcctgaagattttgcaacttattactgtcaacagcttaatagttacccattcactttcggccctgggaccaaagtggatatcaaa

SEQ ID NO: 162 - protein, 107 aa, Artificial Sequence
  synthetic
DIQLTQSPSFLSASVGDRVTITCWASQGISSYLAWYQQKPGKAPKLLIHTASTLQSGVPSRFSGSGSGTEFTLTISNLQPEDFATYYCQQLNSYPFTFGPGTKVDIK

SEQ ID NO: 163 - DNA, 18 bp, Artificial Sequence
  synthetic
cagggcattagcagttat

SEQ ID NO: 164 - protein, 6 aa, Artificial Sequence
  synthetic
QGISSY

SEQ ID NO: 165 - DNA, 9 bp, Artificial Sequence
  synthetic
actgcatcc

SEQ ID NO: 166 - protein, 3 aa, Artificial Sequence
  synthetic
TAS

SEQ ID NO: 167 - DNA, 27 bp, Artificial Sequence
  synthetic
caacagcttaatagttacccattcact

SEQ ID NO: 168 - protein, 9 aa, Artificial Sequence
  synthetic
QQLNSYPFT

SEQ ID NO: 169 - DNA, 366 bp, Artificial Sequence
  synthetic
caggtgcagctggtggagtctgggggaggcgtggtccagcctggggggtccctgagactctcctgtgcagcctctggattcaccttcggtggccatgccatgcactgggtccgccaggctccaggcaaggggctggagtggctggcagttatatcatctgatggcagtaataaacagtatgcagattctgtgaagggccgattcaccatctccagggacaatcccaagaacacgctgtatctgcaaatgaacagtctgagagttggggacacggctatttattactgtgcgaaagaggtggcacctcgttattattattacggtctggacgtctggggccaagggaccacggtcaccgtctcctca

SEQ ID NO: 170 - protein, 122 aa, Artificial Sequence
  synthetic
QVQLVESGGGVVQPGGSLRLSCAASGFTFGGHAMHWVRQAPGKGLEWLAVISSDGSNKQYADSVKGRFTISRDNPKNTLYLQMNSLRVGDTAIYYCAKEVAPRYYYYGLDVWGQGTTVTVSS

SEQ ID NO: 171 - DNA, 24 bp, Artificial Sequence
  synthetic
ggattcaccttcggtggccatgcc

SEQ ID NO: 172 - protein, 8 aa, Artificial Sequence
  synthetic
GFTFGGHA

SEQ ID NO: 173 - DNA, 24 bp, Artificial Sequence
  synthetic
atatcatctgatggcagtaataaa

SEQ ID NO: 174 - protein, 8 aa, Artificial Sequence
  synthetic
ISSDGSNK

SEQ ID NO: 175 - DNA, 45 bp, Artificial Sequence
  synthetic
gcgaaagaggtggcacctcgttattattattacggtctggacgtc

SEQ ID NO: 176 - protein, 15 aa, Artificial Sequence
  synthetic
AKEVAPRYYYYGLDV

SEQ ID NO: 177 - DNA, 318 bp, Artificial Sequence
  synthetic
gacatccagatgacccagtctccatcctccctgtctgcatctgtgggagacagagtcaccatcacttgccgggcgagtcaggacattagcaattttttagcctggtatcagcagaaaccagggaaggttcctaaactcctgatctatactgcatccactttacaatcaggggtcccatctcggttcagtggcagtggatctgggacagatttcactctcaccgtcagcagcctacagcctgaagatgttgcaacttattactgtcaaaagtatgccggcgccctcactttcggccctgggaccaaagtggatatcaaa

SEQ ID NO: 178 - protein, 106 aa, Artificial Sequence
  synthetic
DIQMTQSPSSLSASVGDRVTITCRASQDISNFLAWYQQKPGKVPKLLIYTASTLQSGVPSRFSGSGSGTDFTLTVSSLQPEDVATYYCQKYAGALTFGPGTKVDIK

SEQ ID NO: 179 - DNA, 18 bp, Artificial Sequence
  synthetic
caggacattagcaatttt

SEQ ID NO: 180 - protein, 6 aa, Artificial Sequence
  synthetic
QDISNF

SEQ ID NO: 181 - DNA, 9 bp, Artificial Sequence
  synthetic
actgcatcc

SEQ ID NO: 182 - protein, 3 aa, Artificial Sequence
  synthetic
TAS

SEQ ID NO: 183 - DNA, 24 bp, Artificial Sequence
  synthetic
caaaagtatgccggcgccctcact

SEQ ID NO: 184 - protein, 8 aa, Artificial Sequence
  synthetic
QKYAGALT

SEQ ID NO: 185 - DNA, 357 bp, Artificial Sequence
  synthetic
gaggtgcagctggtggagtctgggggaggcttggcacagcctggggggtccctgagactctcctgtgcagcctctggattcacgtttagaagctatgccatgagctgggtccgccaggctccagggaaggggccggagtgggtctcaggtataggtggtaatggtgttaccacatactacgcagactccgtgaagggccggttcaccatctccagagacaattccaagaacacgctgtttctgcaaatgaatagcctgagagccgaggacacggccgtatattattgtgtgcaggggggtttaggtggttattttacaggctactggggccagggaaccctggtcaccgtctcctca

SEQ ID NO: 186 - protein, 119 aa, Artificial Sequence
  synthetic
EVQLVESGGGLAQPGGSLRLSCAASGFTFRSYAMSWVRQAPGKGPEWVSGIGGNGVTTYYADSVKGRFTISRDNSKNTLFLQMNSLRAEDTAVYYCVQGGLGGYFTGYWGQGTLVTVSS

SEQ ID NO: 187 - DNA, 24 bp, Artificial Sequence
  synthetic
ggattcacgtttagaagctatgcc

SEQ ID NO: 188 - protein, 8 aa, Artificial Sequence
  synthetic
GFTFRSYA

SEQ ID NO: 189 - DNA, 24 bp, Artificial Sequence
  synthetic
ataggtggtaatggtgttaccaca

SEQ ID NO: 190 - protein, 8 aa, Artificial Sequence
  synthetic
IGGNGVTT

SEQ ID NO: 191 - DNA, 36 bp, Artificial Sequence
  synthetic
gtgcaggggggtttaggtggttattttacaggctac

SEQ ID NO: 192 - protein, 12 aa, Artificial Sequence
  synthetic
VQGGLGGYFTGY

SEQ ID NO: 193 - DNA, 321 bp, Artificial Sequence
  synthetic
gacatccagatgacccagtctccatcctccctgtctgcatctgtaggagacagagtcaccatcacttgccgggcaagtcagagtattagtacctatttaaattggtatcagcagaatccagggaaagcccctaaactcctgatctttgatgcatccagtttgcaaagtggggtcccatcaaggttcagtggcagtggatctgggacagatttcactctcaccatcagaggtctgcaacctgaagattttgcaacttactactgtcaacagagttacagtgccccgctcactttcggcggagggaccaaggtggagatcaaa

SEQ ID NO: 194 - protein, 107 aa, Artificial Sequence
  synthetic
DIQMTQSPSSLSASVGDRVTITCRASQSISTYLNWYQQNPGKAPKLLIFDASSLQSGVPSRFSGSGSGTDFTLTIRGLQPEDFATYYCQQSYSAPLTFGGGTKVEIK

SEQ ID NO: 195 - DNA, 18 bp, Artificial Sequence
  synthetic
cagagtattagtacctat

SEQ ID NO: 196 - protein, 6 aa, Artificial Sequence
  synthetic
QSISTY

SEQ ID NO: 197 - DNA, 9 bp, Artificial Sequence
  synthetic
gatgcatcc

SEQ ID NO: 198 - protein, 3 aa, Artificial Sequence
  synthetic
DAS

SEQ ID NO: 199 - DNA, 27 bp, Artificial Sequence
  synthetic
caacagagttacagtgccccgctcact

SEQ ID NO: 200 - protein, 9 aa, Artificial Sequence
  synthetic
QQSYSAPLT

SEQ ID NO: 201 - DNA, 357 bp, Artificial Sequence
  synthetic
caggtgcagctggtggagtctgggggaggcgtggtccagcctgggaggtccctgagactctcctgtgcagcgtctggattcaccttcagtggttatggcatgcactgggtccgccaggctccaggcaaggggctggagtgggtggcacttatatggcttgatggaagtaatgactactatgcagactccgtgaagggccgattcaccatctccagagacaattccaagaacacgttatatctgcaaatgaacagactgagagccgaggacacggctgtgtattactgtgcgagagatggcccggttgctgctatacccgactactggggccagggaaccctggtcaccgtctcctca

SEQ ID NO: 202 - protein, 119 aa, Artificial Sequence
  synthetic
QVQLVESGGGVVQPGRSLRLSCAASGFTFSGYGMHWVRQAPGKGLEWVALIWLDGSNDYYADSVKGRFTISRDNSKNTLYLQMNRLRAEDTAVYYCARDGPVAAIPDYWGQGTLVTVSS

SEQ ID NO: 203 - DNA, 24 bp, Artificial Sequence
  synthetic
ggattcaccttcagtggttatggc

SEQ ID NO: 204 - protein, 8 aa, Artificial Sequence
  synthetic
GFTFSGYG

SEQ ID NO: 205 - DNA, 24 bp, Artificial Sequence
  synthetic
atatggcttgatggaagtaatgac

SEQ ID NO: 206 - protein, 8 aa, Artificial Sequence
  synthetic
IWLDGSND

SEQ ID NO: 207 - DNA, 36 bp, Artificial Sequence
  synthetic
gcgagagatggcccggttgctgctatacccgactac

SEQ ID NO: 208 - protein, 12 aa, Artificial Sequence
  synthetic
ARDGPVAAIPDY

SEQ ID NO: 209 - DNA, 321 bp, Artificial Sequence
  synthetic
gacatccagatgacccagtctccttccaccctgtctgcatctgtaggagacagagtcaccatcacttgccgggccagtcagagtattagtaggtggttggcctggtatcagctgaaaccagggaaagcccctaagctcctgatctataaggcgtctagtttagaaagtggggtcccatcaaggttcagcggcagtggatctgggacagacttcactctcaccatcagcagcctgcaacctgatgattttgcaacttattactgccaacagtataatacttattcgtacacttttggccaggggaccaagctggagatcaaa

SEQ ID NO: 210 - protein, 107 aa, Artificial Sequence
  synthetic
DIQMTQSPSTLSASVGDRVTITCRASQSISRWLAWYQLKPGKAPKLLIYKASSLESGVPSRFSGSGSGTDFTLTISSLQPDDFATYYCQQYNTYSYTFGQGTKLEIK

SEQ ID NO: 211 - DNA, 18 bp, Artificial Sequence
  synthetic
cagagtattagtaggtgg

SEQ ID NO: 212 - protein, 6 aa, Artificial Sequence
  synthetic
QSISRW

SEQ ID NO: 213 - DNA, 9 bp, Artificial Sequence
  synthetic
aaggcgtct

SEQ ID NO: 214 - protein, 3 aa, Artificial Sequence
  synthetic
KAS

SEQ ID NO: 215 - DNA, 27 bp, Artificial Sequence
  synthetic
caacagtataatacttattcgtacact

SEQ ID NO: 216 - protein, 9 aa, Artificial Sequence
  synthetic
QQYNTYSYT

SEQ ID NO: 217 - DNA, 363 bp, Artificial Sequence
  synthetic
gaggtgcagctggtggagtctgggggaggtgtggtacggcctggggggtccctgagactctcctgtgcagcctctggattcacctttgatgaatatggcatgacttgggtccgccaagttccagggaaggggctggagtgggtctctggtattacttggaatggtggtttcacagattatacagactctgtgaagggccgattcaccagctccagagacaacgccaagaactccctgtatctgcaaatgaacagtctgagagccgaggacacggccttgtattactgtgcgagagatggatatagcagctcgtggggggcttatgatatatggggccaagggacaatggtcaccgtctcttca

SEQ ID NO: 218 - protein, 121 aa, Artificial Sequence
  synthetic
EVQLVESGGGVVRPGGSLRLSCAASGFTFDEYGMTWVRQVPGKGLEWVSGITWNGGFTDYTDSVKGRFTSSRDNAKNSLYLQMNSLRAEDTALYYCARDGYSSSWGAYDIWGQGTMVTVSS

SEQ ID NO: 219 - DNA, 24 bp, Artificial Sequence
  synthetic
ggattcacctttgatgaatatggc

SEQ ID NO: 220 - protein, 8 aa, Artificial Sequence
  synthetic
GFTFDEYG

SEQ ID NO: 221 - DNA, 24 bp, Artificial Sequence
  synthetic
attacttggaatggtggtttcaca

SEQ ID NO: 222 - protein, 8 aa, Artificial Sequence
  synthetic
ITWNGGFT

SEQ ID NO: 223 - DNA, 42 bp, Artificial Sequence
  synthetic
gcgagagatggatatagcagctcgtggggggcttatgatata

SEQ ID NO: 224 - protein, 14 aa, Artificial Sequence
  synthetic
ARDGYSSSWGAYDI

SEQ ID NO: 225 - DNA, 321 bp, Artificial Sequence
  synthetic
gacatccagatgacccagtctccatcatccctgtctgcatctgtgggagacagagtcaccatcacttgccgggcaagtcagagcattagcacctatttaaattggtatcagcagaaaccagggaaagcccctaagctcctgatctatgctgcatccagtttgcaaagtggggtcccattaaggttcagtggcagtggatctgggactgatttcactctcaccatcagcagtctgcaacctgaagattttgcaagttatttctgtcaacagagttacagtaccccgtacacttttggccaggggaccaagctggagatcaaa

SEQ ID NO: 226 - protein, 107 aa, Artificial Sequence
  synthetic
DIQMTQSPSSLSASVGDRVTITCRASQSISTYLNWYQQKPGKAPKLLIYAASSLQSGVPLRFSGSGSGTDFTLTISSLQPEDFASYFCQQSYSTPYTFGQGTKLEIK

SEQ ID NO: 227 - DNA, 18 bp, Artificial Sequence
  synthetic
cagagcattagcacctat

SEQ ID NO: 228 - protein, 6 aa, Artificial Sequence
  synthetic
QSISTY

SEQ ID NO: 229 - DNA, 9 bp, Artificial Sequence
  synthetic
gctgcatcc

SEQ ID NO: 230 - protein, 3 aa, Artificial Sequence
  synthetic
AAS

SEQ ID NO: 231 - DNA, 27 bp, Artificial Sequence
  synthetic
caacagagttacagtaccccgtacact

SEQ ID NO: 232 - protein, 9 aa, Artificial Sequence
  synthetic
QQSYSTPYT

SEQ ID NO: 233 - DNA, 360 bp, Artificial Sequence
  synthetic
gaagtgcagctggtggagtctgggggaggcgtggtacagcctggggggtccctgagactctcctgtgcagcctctggattcacctttaatgattatgccatgcactgggtccgtcaagctccagggaagggtctggagtgggtctctcttattagtggagatggtggtaacacatactatgcagactctgtgaagggccgactcaccatctccagagacaacagcaaaaactccctgtatctgcaaatgaacagtctgagaacagaggacaccgccttatattactgtgcaaaagataagggctggaacttcggttacttcgatctctggggccgtggcaccctggtcactgtctcctca

SEQ ID NO: 234 - protein, 120 aa, Artificial Sequence
  synthetic
EVQLVESGGGVVQPGGSLRLSCAASGFTFNDYAMHWVRQAPGKGLEWVSLISGDGGNTYYADSVKGRLTISRDNSKNSLYLQMNSLRTEDTALYYCAKDKGWNFGYFDLWGRGTLVTVSS

SEQ ID NO: 235 - DNA, 24 bp, Artificial Sequence
  synthetic
ggattcacctttaatgattatgcc

SEQ ID NO: 236 - protein, 8 aa, Artificial Sequence
  synthetic
GFTFNDYA

SEQ ID NO: 237 - DNA, 24 bp, Artificial Sequence
  synthetic
attagtggagatggtggtaacaca

SEQ ID NO: 238 - protein, 8 aa, Artificial Sequence
  synthetic
ISGDGGNT

SEQ ID NO: 239 - DNA, 39 bp, Artificial Sequence
  synthetic
gcaaaagataagggctggaacttcggttacttcgatctc

SEQ ID NO: 240 - protein, 13 aa, Artificial Sequence
  synthetic
AKDKGWNFGYFDL

SEQ ID NO: 241 - DNA, 327 bp, Artificial Sequence
  synthetic
gacatccagatgacccagtctccatcctccctgtctacatctgtgggagacagagtcaccatcacttgccgggcaagtcagaacattgacacctatttaaattggtatcagcagaaaccagggaaagcccctaaactcctgatctatgatgcatccagtttacaaagtggggtcccatcacggttcagtggcagcggatctgggacagatttcactctcaccatcaccagtctgcaacctgaagattttgccacttactactgtcaacagaatgacaatattcttcaccctctcactttcggcggagggaccaaggtggagatcaaa

SEQ ID NO: 242 - protein, 109 aa, Artificial Sequence
  synthetic
DIQMTQSPSSLSTSVGDRVTITCRASQNIDTYLNWYQQKPGKAPKLLIYDASSLQSGVPSRFSGSGSGTDFTLTITSLQPEDFATYYCQQNDNILHPLTFGGGTKVEIK

SEQ ID NO: 243 - DNA, 18 bp, Artificial Sequence
  synthetic
cagaacattgacacctat

SEQ ID NO: 244 - protein, 6 aa, Artificial Sequence
  synthetic
QNIDTY

SEQ ID NO: 245 - DNA, 9 bp, Artificial Sequence
  synthetic
gatgcatcc

SEQ ID NO: 246 - protein, 3 aa, Artificial Sequence
  synthetic
DAS

SEQ ID NO: 247 - DNA, 33 bp, Artificial Sequence
  synthetic
caacagaatgacaatattcttcaccctctcact

SEQ ID NO: 248 - protein, 11 aa, Artificial Sequence
  synthetic
QQNDNILHPLT

SEQ ID NO: 249 - DNA, 369 bp, Artificial Sequence
  synthetic
gaggtgcagctggtggagtctgggggaggcttggtccaaccgggggggtccctgagactctcctgtgcagcctctggattccactctaatagatattggatggactgggtccgccaggctccagggaaggggctggagtgggtggccaacataaagcaagatggaagtgaggaaaactatgtggactctgtgaagggccgattcaccatctccagagacaacgccaagaactcactttatctgcaaatgaacagcctgagagccgaggacacggctgtgtattactgtgcgagagatcgaagcacctcgtgggtcccttactggttcttcgatctctggggccgtggcaccctggtcactgtctcctca

SEQ ID NO: 250 - protein, 123 aa, Artificial Sequence
  synthetic
EVQLVESGGGLVQPGGSLRLSCAASGFHSNRYWMDWVRQAPGKGLEWVANIKQDGSEENYVDSVKGRFTISRDNAKNSLYLQMNSLRAEDTAVYYCARDRSTSWVPYWFFDLWGRGTLVTVSS

SEQ ID NO: 251 - DNA, 24 bp, Artificial Sequence
  synthetic
ggattccactctaatagatattgg

SEQ ID NO: 252 - protein, 8 aa, Artificial Sequence
  synthetic
GFHSNRYW

SEQ ID NO: 253 - DNA, 24 bp, Artificial Sequence
  synthetic
ataaagcaagatggaagtgaggaa

SEQ ID NO: 254 - protein, 8 aa, Artificial Sequence
  synthetic
IKQDGSEE

SEQ ID NO: 255 - DNA, 48 bp, Artificial Sequence
  synthetic
gcgagagatcgaagcacctcgtgggtcccttactggttcttcgatctc

SEQ ID NO: 256 - protein, 16 aa, Artificial Sequence
  synthetic
ARDRSTSWVPYWFFDL

SEQ ID NO: 257 - DNA, 324 bp, Artificial Sequence
  synthetic
gacatccagatgacccagtctccatcctccctgtctgcatctgtaggagacagagtcaccatcacttgccgggcaagtcagagcattagcagctatttaaattggtatcagcagaaaccagggaaagcccctaagctcctgatctatgctgcatccagtttgcaaagtggggtcccgtcaaggttcagtggcagtggatctgggacagatttcactctcaccatcagcagtctgcaacctgaagattttgcaacttactactgtcaacagagttacagtacccctccgatcaccttcggccaagggacacgactggagattaaa

SEQ ID NO: 258 - protein, 108 aa, Artificial Sequence
  synthetic
DIQMTQSPSSLSASVGDRVTITCRASQSISSYLNWYQQKPGKAPKLLIYAASSLQSGVPSRFSGSGSGTDFTLTISSLQPEDFATYYCQQSYSTPPITFGQGTRLEIK

SEQ ID NO: 259 - DNA, 18 bp, Artificial Sequence
  synthetic
cagagcattagcagctat

SEQ ID NO: 260 - protein, 6 aa, Artificial Sequence
  synthetic
QSISSY

SEQ ID NO: 261 - DNA, 9 bp, Artificial Sequence
  synthetic
gctgcatcc

SEQ ID NO: 262 - protein, 3 aa, Artificial Sequence
  synthetic
AAS

SEQ ID NO: 263 - DNA, 30 bp, Artificial Sequence
  synthetic
caacagagttacagtacccctccgatcacc

SEQ ID NO: 264 - protein, 10 aa, Artificial Sequence
  synthetic
QQSYSTPPIT

SEQ ID NO: 265 - DNA, 360 bp, Artificial Sequence
  synthetic
gaagtgcagctggtggagtctgggggaggcgtggtacagcggggggagtccctgagactctcctgttcagcctctgacttcatctttaaagattatgccatgtactgggtccgtcaaattccagggaagggtctagagtggatctctcttattagtggtgatggtgacactacatggtatggagactctgtgaagggccgattcaccatctccagagacaacaacgaaaactccctctttctgcaaatgaacgatctgagaactgaggacaccgccatgtactactgtgcaagagatatggggtggaacttctttcagttgcaatactggggccagggaaccctggtcaccgtctcctca

SEQ ID NO: 266 - protein, 120 aa, Artificial Sequence
  synthetic
EVQLVESGGGVVQRGESLRLSCSASDFIFKDYAMYWVRQIPGKGLEWISLISGDGDTTWYGDSVKGRFTISRDNNENSLFLQMNDLRTEDTAMYYCARDMGWNFFQLQYWGQGTLVTVSS

SEQ ID NO: 267 - DNA, 24 bp, Artificial Sequence
  synthetic
gacttcatctttaaagattatgcc

SEQ ID NO: 268 - protein, 8 aa, Artificial Sequence
  synthetic
DFIFKDYA

SEQ ID NO: 269 - DNA, 24 bp, Artificial Sequence
  synthetic
attagtggtgatggtgacactaca

SEQ ID NO: 270 - protein, 8 aa, Artificial Sequence
  synthetic
ISGDGDTT

SEQ ID NO: 271 - DNA, 39 bp, Artificial Sequence
  synthetic
gcaagagatatggggtggaacttctttcagttgcaatac

SEQ ID NO: 272 - protein, 13 aa, Artificial Sequence
  synthetic
ARDMGWNFFQLQY

SEQ ID NO: 273 - DNA, 361 bp, Artificial Sequence
  synthetic
dcaggtgcagctgcaggagtcgggccccgcactggtgaagccttcacagaccctgtccctcacctgcactgtctctggtggctccatcatcagaggtagtacctactggagttgggtccgccaattcccagggaagggcctggagtggattggatacagttattacagtgggaccgcctactataatccgtccctcgagagtcgagctaccatttctgtagacacgtctaagaaccagttctccctgaacctgaagtctgtgacggccgcggacacggccgtgtattattgtacaagagaaataggagtggctggtctctttgacatctggggccagggaaccctggtcaccgtctcctca

SEQ ID NO: 274 - protein, 120 aa, Artificial Sequence
  synthetic
QVQLQESGPALVKPSQTLSLTCTVSGGSIIRGSTYWSWVRQFPGKGLEWIGYSYYSGTAYYNPSLESRATISVDTSKNQFSLNLKSVTAADTAVYYCTREIGVAGLFDIWGQGTLVTVSS

SEQ ID NO: 275 - DNA, 30 bp, Artificial Sequence
  synthetic
ggtggctccatcatcagaggtagtacctac

SEQ ID NO: 276 - protein, 10 aa, Artificial Sequence
  synthetic
GGSIIRGSTY

SEQ ID NO: 277 - DNA, 21 bp, Artificial Sequence
  synthetic
agttattacagtgggaccgcc

SEQ ID NO: 278 - protein, 7 aa, Artificial Sequence
  synthetic
SYYSGTA

SEQ ID NO: 279 - DNA, 36 bp, Artificial Sequence
  synthetic
acaagagaaataggagtggctggtctctttgacatc

SEQ ID NO: 280 - protein, 12 aa, Artificial Sequence
  synthetic
TREIGVAGLFDI

SEQ ID NO: 281 - DNA, 324 bp, Artificial Sequence
  synthetic
gaaatagttttgacacagagtcccggcacactgtcactctctcccggggaaagagccaccttgtcatgtagagcaagtcagtcagtctctagctcttatctcgcctggtaccagcagaagccgggacaggcccctagactgctgatctacggggcaagttccagggccaccggaatccccgaccggttcagtggaagcggaagcggaaccgattttactttgacgatttctagactggagccagaggatttcgccgtttactattgtcaacagtacggaagcagcccgtggacgtttggccagggcacgaaggtagaaatcaag

SEQ ID NO: 282 - protein, 108 aa, Artificial Sequence
  synthetic
EIVLTQSPGTLSLSPGERATLSCRASQSVSSSYLAWYQQKPGQAPRLLIYGASSRATGIPDRFSGSGSGTDFTLTISRLEPEDFAVYYCQQYGSSPWTFGQGTKVEIK

SEQ ID NO: 283 - DNA, 36 bp, Artificial Sequence
  synthetic
agagcaagtcagtcagtctctagctcttatctcgcc

SEQ ID NO: 284 - protein, 12 aa, Artificial Sequence
  synthetic
RASQSVSSSYLA

SEQ ID NO: 285 - DNA, 21 bp, Artificial Sequence
  synthetic
ggggcaagttccagggccacc

SEQ ID NO: 286 - protein, 7 aa, Artificial Sequence
  synthetic
GASSRAT

SEQ ID NO: 287 - DNA, 27 bp, Artificial Sequence
  synthetic
caacagtacggaagcagcccgtggacg

SEQ ID NO: 288 - protein, 9 aa, Artificial Sequence
  synthetic
QQYGSSPWT

SEQ ID NO: 289 - DNA, 357 bp, Artificial Sequence
  synthetic
caggagcagttggtgcagtctggggctgaggtgaagaagcctggggcctcagtgaaggtctcctgtaaggcttctggatacaccttcaccggctactatatacattgggtgcgacaggcccctggactagggcttgaatggatgggatggatcaaccctaacagtggtggcacaaaatatgcacagaagtttcagggcagggtcaccatgaccagggacacgtccatcaatacagcctacatggagctgaaaagactgaaatctgacgactcggccgtatattactgtgcgagagacgcccctccccatgatgtttttgatatctggggccaagggacattggtcaccgtctcttca

SEQ ID NO: 290 - protein, 119 aa, Artificial Sequence
  synthetic
QEQLVQSGAEVKKPGASVKVSCKASGYTFTGYYIHWVRQAPGLGLEWMGWINPNSGGTKYAQKFQGRVTMTRDTSINTAYMELKRLKSDDSAVYYCARDAPPHDVFDIWGQGTLVTVSS

SEQ ID NO: 291 - DNA, 24 bp, Artificial Sequence
  synthetic
ggatacaccttcaccggctactat

SEQ ID NO: 292 - protein, 8 aa, Artificial Sequence
  synthetic
GYTFTGYY

SEQ ID NO: 293 - DNA, 24 bp, Artificial Sequence
  synthetic
atcaaccctaacagtggtggcaca

SEQ ID NO: 294 - protein, 8 aa, Artificial Sequence
  synthetic
INPNSGGT

SEQ ID NO: 295 - DNA, 36 bp, Artificial Sequence
  synthetic
gcgagagacgcccctccccatgatgtttttgatatc

SEQ ID NO: 296 - protein, 12 aa, Artificial Sequence
  synthetic
ARDAPPHDVFDI

SEQ ID NO: 297 - DNA, 321 bp, Artificial Sequence
  synthetic
gacatccagatgacccagtctccatcctccctgtctgcatctgtaggagacagagtcaccatcacttgccgggcaagtcagggcattagaaatgatttaggctggtatcagcagaaaccagggaaagcccctaagcgcctgatctatgctgcatccagtttgcaaattggggtcccatcaaggttcagcggcagtggatctgggacagaattcactctcacaatcagcagcctgcagcctgaagattttgcaacttattactgtctacagcataatagttacccgctcactttcggcggagggaccaaggtggagatcaaa

SEQ ID NO: 298 - protein, 107 aa, Artificial Sequence
  synthetic
DIQMTQSPSSLSASVGDRVTITCRASQGIRNDLGWYQQKPGKAPKRLIYAASSLQIGVPSRFSGSGSGTEFTLTISSLQPEDFATYYCLQHNSYPLTFGGGTKVEIK

SEQ ID NO: 299 - DNA, 18 bp, Artificial Sequence
  synthetic
cagggcattagaaatgat

SEQ ID NO: 300 - protein, 6 aa, Artificial Sequence
  synthetic
QGIRND

SEQ ID NO: 301 - DNA, 9 bp, Artificial Sequence
  synthetic
gctgcatcc

SEQ ID NO: 302 - protein, 3 aa, Artificial Sequence
  synthetic
AAS

SEQ ID NO: 303 - DNA, 27 bp, Artificial Sequence
  synthetic
ctacagcataatagttacccgctcact

SEQ ID NO: 304 - protein, 9 aa, Artificial Sequence
  synthetic
LQHNSYPLT

SEQ ID NO: 305 - DNA, 357 bp, Artificial Sequence
  synthetic
caggtgcagctgcaagagtcgggcccaggactggtgaagccttcacagaccctgtccctcacctgcactgtctctggtggctccatcagtagtggtgcttaccactggagctggatccgccagcacccagggaagggcctagagtggattggatacatctattacaatggggacacctactataatccgtccctcaagagtcgcgttaccatttcagtggacacgtctaagaaccaattcttcctgaaggtgacctctgtgactgccgcggacacggccatgtattactgtgcgggagaaaagcagctgactgcttttgatatctggggccaagggacattggtcaccgtctcttca

SEQ ID NO: 306 - protein, 119 aa, Artificial Sequence
  synthetic
QVQLQESGPGLVKPSQTLSLTCTVSGGSISSGAYHWSWIRQHPGKGLEWIGYIYYNGDTYYNPSLKSRVTISVDTSKNQFFLKVTSVTAADTAMYYCAGEKQLTAFDIWGQGTLVTVSS

SEQ ID NO: 307 - DNA, 30 bp, Artificial Sequence
  synthetic
ggtggctccatcagtagtggtgcttaccac

SEQ ID NO: 308 - protein, 10 aa, Artificial Sequence
  synthetic
GGSISSGAYH

SEQ ID NO: 309 - DNA, 21 bp, Artificial Sequence
  synthetic
atctattacaatggggacacc

SEQ ID NO: 310 - protein, 7 aa, Artificial Sequence
  synthetic
IYYNGDT

SEQ ID NO: 311 - DNA, 33 bp, Artificial Sequence
  synthetic
gcgggagaaaagcagctgactgcttttgatatc

SEQ ID NO: 312 - protein, 11 aa, Artificial Sequence
  synthetic
AGEKQLTAFDI

SEQ ID NO: 313 - DNA, 321 bp, Artificial Sequence
  synthetic
gtcatccagatgacccagtctccatcctccctgtctgcatctgttggagacagagtcaccataacttgccgggcgagtcaggacattaataattttttaaattggtatcaacagaaattagggaaagcccctaaactcctgatctccgatgcatccaatttgcagacaggagtcccgtcaaggttcagtggaagtggatctgggacagattttactttcaccatcagcagcctgcagcctgaagatattgctgcatattactgtcaacaatatgatcatttcccgtatacttttggccaggggaccagactggagaacaat

SEQ ID NO: 314 - protein, 107 aa, Artificial Sequence
  synthetic
VIQMTQSPSSLSASVGDRVTITCRASQDINNFLNWYQQKLGKAPKLLISDASNLQTGVPSRFSGSGSGTDFTFTISSLQPEDIAAYYCQQYDHFPYTFGQGTRLENN

SEQ ID NO: 315 - DNA, 18 bp, Artificial Sequence
  synthetic
caggacattaataatttt

SEQ ID NO: 316 - protein, 6 aa, Artificial Sequence
  synthetic
QDINNF

SEQ ID NO: 317 - DNA, 9 bp, Artificial Sequence
  synthetic
gatgcatcc

SEQ ID NO: 318 - protein, 3 aa, Artificial Sequence
  synthetic
DAS

SEQ ID NO: 319 - DNA, 27 bp, Artificial Sequence
  synthetic
caacaatatgatcatttcccgtatact

SEQ ID NO: 320 - protein, 9 aa, Artificial Sequence
  synthetic
QQYDHFPYT

SEQ ID NO: 321 - DNA, 357 bp, Artificial Sequence
  synthetic
gaggtgcagttggtggagtctgggggaggtgtggttcggcctggggggtccctgagactctcctgtgcagcctctggattcacctttgatgattatggcatgacctgggtccgccaagctccagggaaggggctggagtgggtctctggtattaattggaatggcgatagcacagagtattcagactctgtgaagggccgattcaccatctccagagacaacgccaagaactccctgtatctgcaaatgaacagtctgagagccgaggacacggccttctatcactgtgcgagagagaataactggaacttctactttgactactggggccagggaaccctggtcaccgtctcctca

SEQ ID NO: 322 - protein, 119 aa, Artificial Sequence
  synthetic
EVQLVESGGGVVRPGGSLRLSCAASGFTFDDYGMTWVRQAPGKGLEWVSGINWNGDSTEYSDSVKGRFTISRDNAKNSLYLQMNSLRAEDTAFYHCARENNWNFYFDYWGQGTLVTVSS

SEQ ID NO: 323 - DNA, 24 bp, Artificial Sequence
  synthetic
ggattcacctttgatgattatggc

SEQ ID NO: 324 - protein, 8 aa, Artificial Sequence
  synthetic
GFTFDDYG

SEQ ID NO: 325 - DNA, 24 bp, Artificial Sequence
  synthetic
attaattggaatggcgatagcaca

SEQ ID NO: 326 - protein, 8 aa, Artificial Sequence
  synthetic
INWNGDST

SEQ ID NO: 327 - DNA, 36 bp, Artificial Sequence
  synthetic
gcgagagagaataactggaacttctactttgactac

SEQ ID NO: 328 - protein, 12 aa, Artificial Sequence
  synthetic
ARENNWNFYFDY

SEQ ID NO: 329 - DNA, 321 bp, Artificial Sequence
  synthetic
gaaatagtgatgacgcagtctccagccaccctgtctgtgtctcgaggggaaagagccaccctctcctgtagggccagtcagagtgttagcagcaacttagcctggtaccagcagaaacttggccaggctcccaggctcctcatctatggtgcatccaccagggccactggtatcccagccaggttcagtggcagtgggtctgggacagagttcactctcaccatcagcagcctgcagtctgaagattttgcagtttattattgtcagcagtataataactggccgtggacgttcggccaagggaccaaggtggaaatcaaa

SEQ ID NO: 330 - protein, 107 aa, Artificial Sequence
  synthetic
EIVMTQSPATLSVSRGERATLSCRASQSVSSNLAWYQQKLGQAPRLLIYGASTRATGIPARFSGSGSGTEFTLTISSLQSEDFAVYYCQQYNNWPWTFGQGTKVEIK

SEQ ID NO: 331 - DNA, 18 bp, Artificial Sequence
  synthetic
cagagtgttagcagcaac

SEQ ID NO: 332 - protein, 6 aa, Artificial Sequence
  synthetic
QSVSSN

SEQ ID NO: 333 - DNA, 9 bp, Artificial Sequence
  synthetic
ggtgcatcc

SEQ ID NO: 334 - protein, 3 aa, Artificial Sequence
  synthetic
GAS

SEQ ID NO: 335 - DNA, 27 bp, Artificial Sequence
  synthetic
cagcagtataataactggccgtggacg

SEQ ID NO: 336 - protein, 9 aa, Artificial Sequence
  synthetic
QQYNNWPWT

SEQ ID NO: 337 - DNA, 351 bp, Artificial Sequence
  synthetic
caggtccacctggtacagtctggggctgaggtgaagaagcctggggcctcagtgaaggtctcctgcaaggtttccggaaacaccctcactgaattatccatgcactgggtgcgacaggctcctggaaaagggcttgagtggatgggaggttttgatcctgaagatggtgacacaatctactcacagaagttccagggcagagtcaccttgaccgaggacacatctacagacacagcctacatggagctgagcagcctgagatctgaggacacggccgtgtattactgttcaacagtggggggacctacctctgactgctggggccagggaaccctggtcaccgtctcctca

SEQ ID NO: 338 - protein, 117 aa, Artificial Sequence
  synthetic
QVHLVQSGAEVKKPGASVKVSCKVSGNTLTELSMHWVRQAPGKGLEWMGGFDPEDGDTIYSQKFQGRVTLTEDTSTDTAYMELSSLRSEDTAVYYCSTVGGPTSDCWGQGTLVTVSS

SEQ ID NO: 339 - DNA, 24 bp, Artificial Sequence
  synthetic
ggaaacaccctcactgaattatcc

SEQ ID NO: 340 - protein, 8 aa, Artificial Sequence
  synthetic
GNTLTELS

SEQ ID NO: 341 - DNA, 24 bp, Artificial Sequence
  synthetic
tttgatcctgaagatggtgacaca

SEQ ID NO: 342 - protein, 8 aa, Artificial Sequence
  synthetic
FDPEDGDT

SEQ ID NO: 343 - DNA, 30 bp, Artificial Sequence
  synthetic
tcaacagtggggggacctacctctgactgc

SEQ ID NO: 344 - protein, 10 aa, Artificial Sequence
  synthetic
STVGGPTSDC

SEQ ID NO: 345 - DNA, 321 bp, Artificial Sequence
  synthetic
gacatccagatgacccagtctccatcctccctgtctgcatctgtaggagacagagtcaccatcacttgccaggcgagtcaggacattagcaactatttaaattggtatcagcagaaaccagggaaagcccctaaggtcctgatcttcgatgcatccaatttagaaccaggggtcccatcaaggttcagtggaagtggatctgggacagattttactttcaccatcatcagcctgcagcctgaagatattgcaacatattactgtcaacaatatgataatctcccgatcaccttcggccaggggacacgactggacattaaa

SEQ ID NO: 346 - protein, 107 aa, Artificial Sequence
  synthetic
DIQMTQSPSSLSASVGDRVTITCQASQDISNYLNWYQQKPGKAPKVLIFDASNLEPGVPSRFSGSGSGTDFTFTIISLQPEDIATYYCQQYDNLPITFGQGTRLDIK

SEQ ID NO: 347 - DNA, 18 bp, Artificial Sequence
  synthetic
caggacattagcaactat

SEQ ID NO: 348 - protein, 6 aa, Artificial Sequence
  synthetic
QDISNY

SEQ ID NO: 349 - DNA, 9 bp, Artificial Sequence
  synthetic
gatgcatcc

SEQ ID NO: 350 - protein, 3 aa, Artificial Sequence
  synthetic
DAS

SEQ ID NO: 351 - DNA, 27 bp, Artificial Sequence
  synthetic
caacaatatgataatctcccgatcacc

SEQ ID NO: 352 - protein, 9 aa, Artificial Sequence
  synthetic
QQYDNLPIT

SEQ ID NO: 353 - protein, 447 aa, Artificial Sequence
  HC
QVQLQESGPGLVKPSETLSLTCTVSGDSVSSSYWTWIRQPPGKGLEWIGYIYYSGSSNYNPSLKSRATISVDTSKNQFSLKLSSVTAADTAVYYCAREGNVDTTMIFDYWGQGTLVTVSSASTKGPSVFPLAPCSRSTSESTAALGCLVKDYFPEPVTVSWNSGALTSGVHTFPAVLQSSGLYSLSSVVTVPSSSLGTKTYTCNVDHKPSNTKVDKRVESKYGPPCPPCPAPEFLGGPSVFLFPPKPKDTLMISRTPEVTCVVVDVSQEDPEVQFNWYVDGVEVHNAKTKPREEQFNSTYRVVSVLTVLHQDWLNGKEYKCKVSNKGLPSSIEKTISKAKGQPREPQVYTLPPSQEEMTKNQVSLTCLVKGFYPSDIAVEWESNGQPENNYKTTPPVLDSDGSFFLYSRLTVDKSRWQEGNVFSCSVMHEALHNHYTQKSLSLSLGK

SEQ ID NO: 354 - protein, 214 aa, Artificial Sequence
  LC
AIQMTQSPSSLSASVGDRVTITCRASQGIRNDLGWYQQKPGKAPKLLIYAASSLQSGVPSRFAGRGSGTDFTLTISSLQPEDFATYYCLQDFNYPWTFGQGTKVEIKRTVAAPSVFIFPPSDEQLKSGTASVVCLLNNFYPREAKVQWKVDNALQSGNSQESVTEQDSKDSTYSLSSTLTLSKADYEKHKVYACEVTHQGLSSPVTKSFNRGEC

SEQ ID NO: 355 - protein, 1676 aa, Artificial Sequence
  human C5
MGLLGILCFLIFLGKTWGQEQTYVISAPKIFRVGASENIVIQVYGYTEAFDATISIKSYPDKKFSYSSGHVHLSSENKFQNSAILTIQPKQLPGGQNPVSYVYLEVVSKHFSKSKRMPITYDNGFLFIHTDKPVYTPDQSVKVRVYSLNDDLKPAKRETVLTFIDPEGSEVDMVEEIDHIGIISFPDFKIPSNPRYGMWTIKAKYKEDFSTTGTAYFEVKEYVLPHFSVSIEPEYNFIGYKNFKNFEITIKARYFYNKVVTEADVYITFGIREDLKDDQKEMMQTAMQNTMLINGIAQVTFDSETAVKELSYYSLEDLNNKYLYIAVTVIESTGGFSEEAEIPGIKYVLSPYKLNLVATPLFLKPGIPYPIKVQVKDSLDQLVGGVPVTLNAQTIDVNQETSDLDPSKSVTRVDDGVASFVLNLPSGVTVLEFNVKTDAPDLPEENQAREGYRAIAYSSLSQSYLYIDWTDNHKALLVGEHLNIIVTPKSPYIDKITHYNYLILSKGKIIHFGTREKFSDASYQSINIPVTQNMVPSSRLLVYYIVTGEQTAELVSDSVWLNIEEKCGNQLQVHLSPDADAYSPGQTVSLNMATGMDSWVALAAVDSAVYGVQRGAKKPLERVFQFLEKSDLGCGAGGGLNNANVFHLAGLTFLTNANADDSQENDEPCKEILRPRRTLQKKIEEIAAKYKHSVVKKCCYDGACVNNDETCEQRAARISLGPRCIKAFTECCVVASQLRANISHKDMQLGRLHMKTLLPVSKPEIRSYFPESWLWEVHLVPRRKQLQFALPDSLTTWEIQGVGISNTGICVADTVKAKVFKDVFLEMNIPYSVVRGEQIQLKGTVYNYRTSGMQFCVKMSAVEGICTSESPVIDHQGTKSSKCVRQKVEGSSSHLVTFTVLPLEIGLHNINFSLETWFGKEILVKTLRVVPEGVKRESYSGVTLDPRGIYGTISRRKEFPYRIPLDLVPKTEIKRILSVKGLLVGEILSAVLSQEGINILTHLPKGSAEAELMSVVPVFYVFHYLETGNHWNIFHSDPLIEKQKLKKKLKEGMLSIMSYRNADYSYSVWKGGSASTWLTAFALRVLGQVNKYVEQNQNSICNSLLWLVENYQLDNGSFKENSQYQPIKLQGTLPVEARENSLYLTAFTVIGIRKAFDICPLVKIDTALIKADNFLLENTLPAQSTFTLAISAYALSLGDKTHPQFRSIVSALKREALVKGNPPIYRFWKDNLQHKDSSVPNTGTARMVETTAYALLTSLNLKDINYVNPVIKWLSEEQRYGGGFYSTQDTINAIEGLTEYSLLVKQLRLSMDIDVSYKHKGALHNYKMTDKNFLGRPVEVLLNDDLIVSTGFGSGLATVHVTTVVHKTSTSEEVCSFYLKIDTQDIEASHYRGYGNSDYKRIVACASYKPSREESSSGSSHAVMDISLPTGISANEEDLKALVEGVDQLFTDYQIKDGHVILQLNSIPSSDFLCVRFRIFELFEVGFLSPATFTVYEYHRPDKQCTMFYSTSNIKIQKVCEGAACKCVEADCGQMQEELDLTISAETRKQTACKPEIAYAYKVSITSITVENVFVKYKATLLDIYKTGEAVAEKDSEITFIKKVTCTNAELVKGRQYLIMGKEALQIKYNFSFRYIYPLDSLTWIEYWPRDTTCSSCQAFLANLDEFAEDIFLNGC

SEQ ID NO: 356 - protein, 1686 aa, Artificial Sequence
  hC5 R885H aa 1-1658: hC5 (aa 19-1676 of NM_001735.2 with R885H change) aa 1659-1686: myc-myc-hexahistidine tag
QEQTYVISAPKIFRVGASENIVIQVYGYTEAFDATISIKSYPDKKFSYSSGHVHLSSENKFQNSAILTIQPKQLPGGQNPVSYVYLEVVSKHFSKSKRMPITYDNGFLFIHTDKPVYTPDQSVKVRVYSLNDDLKPAKRETVLTFIDPEGSEVDMVEEIDHIGIISFPDFKIPSNPRYGMWTIKAKYKEDFSTTGTAYFEVKEYVLPHFSVSIEPEYNFIGYKNFKNFEITIKARYFYNKVVTEADVYITFGIREDLKDDQKEMMQTAMQNTMLINGIAQVTFDSETAVKELSYYSLEDLNNKYLYIAVTVIESTGGFSEEAEIPGIKYVLSPYKLNLVATPLFLKPGIPYPIKVQVKDSLDQLVGGVPVTLNAQTIDVNQETSDLDPSKSVTRVDDGVASFVLNLPSGVTVLEFNVKTDAPDLPEENQAREGYRAIAYSSLSQSYLYIDWTDNHKALLVGEHLNIIVTPKSPYIDKITHYNYLILSKGKIIHFGTREKFSDASYQSINIPVTQNMVPSSRLLVYYIVTGEQTAELVSDSVWLNIEEKCGNQLQVHLSPDADAYSPGQTVSLNMATGMDSWVALAAVDSAVYGVQRGAKKPLERVFQFLEKSDLGCGAGGGLNNANVFHLAGLTFLTNANADDSQENDEPCKEILRPRRTLQKKIEEIAAKYKHSVVKKCCYDGACVNNDETCEQRAARISLGPRCIKAFTECCVVASQLRANISHKDMQLGRLHMKTLLPVSKPEIRSYFPESWLWEVHLVPRRKQLQFALPDSLTTWEIQGVGISNTGICVADTVKAKVFKDVFLEMNIPYSVVRGEQIQLKGTVYNYRTSGMQFCVKMSAVEGICTSESPVIDHQGTKSSKCVHQKVEGSSSHLVTFTVLPLEIGLHNINFSLETWFGKEILVKTLRVVPEGVKRESYSGVTLDPRGIYGTISRRKEFPYRIPLDLVPKTEIKRILSVKGLLVGEILSAVLSQEGINILTHLPKGSAEAELMSVVPVFYVFHYLETGNHWNIFHSDPLIEKQKLKKKLKEGMLSIMSYRNADYSYSVWKGGSASTWLTAFALRVLGQVNKYVEQNQNSICNSLLWLVENYQLDNGSFKENSQYQPIKLQGTLPVEARENSLYLTAFTVIGIRKAFDICPLVKIDTALIKADNFLLENTLPAQSTFTLAISAYALSLGDKTHPQFRSIVSALKREALVKGNPPIYRFWKDNLQHKDSSVPNTGTARMVETTAYALLTSLNLKDINYVNPVIKWLSEEQRYGGGFYSTQDTINAIEGLTEYSLLVKQLRLSMDIDVSYKHKGALHNYKMTDKNFLGRPVEVLLNDDLIVSTGFGSGLATVHVTTVVHKTSTSEEVCSFYLKIDTQDIEASHYRGYGNSDYKRIVACASYKPSREESSSGSSHAVMDISLPTGISANEEDLKALVEGVDQLFTDYQIKDGHVILQLNSIPSSDFLCVRFRIFELFEVGFLSPATFTVYEYHRPDKQCTMFYSTSNIKIQKVCEGAACKCVEADCGQMQEELDLTISAETRKQTACKPEIAYAYKVSITSITVENVFVKYKATLLDIYKTGEAVAEKDSEITFIKKVTCTNAELVKGRQYLIMGKEALQIKYNFSFRYIYPLDSLTWIEYWPRDTTCSSCQAFLANLDEFAEDIFLNGCEQKLISEEDLGGEQKLISEEDLHHHHHH

SEQ ID NO: 357 - protein, 1686 aa, Artificial Sequence
  hC5 R885C aa 1-1658: hC5 (aa 19-1676 of NM_001735.2 with R885C change) aa 1659-1686: myc-myc-hexahistidine tag
QEQTYVISAPKIFRVGASENIVIQVYGYTEAFDATISIKSYPDKKFSYSSGHVHLSSENKFQNSAILTIQPKQLPGGQNPVSYVYLEVVSKHFSKSKRMPITYDNGFLFIHTDKPVYTPDQSVKVRVYSLNDDLKPAKRETVLTFIDPEGSEVDMVEEIDHIGIISFPDFKIPSNPRYGMWTIKAKYKEDFSTTGTAYFEVKEYVLPHFSVSIEPEYNFIGYKNFKNFEITIKARYFYNKVVTEADVYITFGIREDLKDDQKEMMQTAMQNTMLINGIAQVTFDSETAVKELSYYSLEDLNNKYLYIAVTVIESTGGFSEEAEIPGIKYVLSPYKLNLVATPLFLKPGIPYPIKVQVKDSLDQLVGGVPVTLNAQTIDVNQETSDLDPSKSVTRVDDGVASFVLNLPSGVTVLEFNVKTDAPDLPEENQAREGYRAIAYSSLSQSYLYIDWTDNHKALLVGEHLNIIVTPKSPYIDKITHYNYLILSKGKIIHFGTREKFSDASYQSINIPVTQNMVPSSRLLVYYIVTGEQTAELVSDSVWLNIEEKCGNQLQVHLSPDADAYSPGQTVSLNMATGMDSWVALAAVDSAVYGVQRGAKKPLERVFQFLEKSDLGCGAGGGLNNANVFHLAGLTFLTNANADDSQENDEPCKEILRPRRTLQKKIEEIAAKYKHSVVKKCCYDGACVNNDETCEQRAARISLGPRCIKAFTECCVVASQLRANISHKDMQLGRLHMKTLLPVSKPEIRSYFPESWLWEVHLVPRRKQLQFALPDSLTTWEIQGVGISNTGICVADTVKAKVFKDVFLEMNIPYSVVRGEQIQLKGTVYNYRTSGMQFCVKMSAVEGICTSESPVIDHQGTKSSKCVCQKVEGSSSHLVTFTVLPLEIGLHNINFSLETWFGKEILVKTLRVVPEGVKRESYSGVTLDPRGIYGTISRRKEFPYRIPLDLVPKTEIKRILSVKGLLVGEILSAVLSQEGINILTHLPKGSAEAELMSVVPVFYVFHYLETGNHWNIFHSDPLIEKQKLKKKLKEGMLSIMSYRNADYSYSVWKGGSASTWLTAFALRVLGQVNKYVEQNQNSICNSLLWLVENYQLDNGSFKENSQYQPIKLQGTLPVEARENSLYLTAFTVIGIRKAFDICPLVKIDTALIKADNFLLENTLPAQSTFTLAISAYALSLGDKTHPQFRSIVSALKREALVKGNPPIYRFWKDNLQHKDSSVPNTGTARMVETTAYALLTSLNLKDINYVNPVIKWLSEEQRYGGGFYSTQDTINAIEGLTEYSLLVKQLRLSMDIDVSYKHKGALHNYKMTDKNFLGRPVEVLLNDDLIVSTGFGSGLATVHVTTVVHKTSTSEEVCSFYLKIDTQDIEASHYRGYGNSDYKRIVACASYKPSREESSSGSSHAVMDISLPTGISANEEDLKALVEGVDQLFTDYQIKDGHVILQLNSIPSSDFLCVRFRIFELFEVGFLSPATFTVYEYHRPDKQCTMFYSTSNIKIQKVCEGAACKCVEADCGQMQEELDLTISAETRKQTACKPEIAYAYKVSITSITVENVFVKYKATLLDIYKTGEAVAEKDSEITFIKKVTCTNAELVKGRQYLIMGKEALQIKYNFSFRYIYPLDSLTWIEYWPRDTTCSSCQAFLANLDEFAEDIFLNGCEQKLISEEDLGGEQKLISEEDLHHHHHH

SEQ ID NO: 358 - protein, 1686 aa, Artificial Sequence
  M. fascicularis C5 R885H aa 1-1658: M. fascicularis C5 (determined in-house; NTBK#12480) aa 1659-1686: myc-myc-hexahistidine tag
QEQTYVISAPKIFRVGASENIVIQVYGYTEAFDATISIKSYPDKKFSYSSGHVHLSSENKFQNSAVLTIQPKQLPGGQNQVSYVYLEVVSKHFSKSKKIPITYDNGFLFIHTDKPVYTPDQSVKVRVYSLNDDLKPAKRETVLTFIDPEGSEIDMVEEIDHIGIISFPDFKIPSNPRYGMWTIQAKYKEDFSTTGTAFFEVKEYVLPHFSVSVEPESNFIGYKNFKNFEITIKARYFYNKVVTEADVYITFGIREDLKDDQKEMMQTAMQNTMLINGIAQVTFDSETAVKELSYYSLEDLNNKYLYIAVTVIESTGGFSEEAEIPGIKYVLSPYKLNLVATPLFLKPGIPYSIKVQVKDALDQLVGGVPVTLNAQTIDVNQETSDLEPRKSVTRVDDGVASFVVNLPSGVTVLEFNVKTDAPDLPDENQAREGYRAIAYSSLSQSYLYIDWTDNHKALLVGEYLNIIVTPKSPYIDKITHYNYLILSKGKIIHFGTREKLSDASYQSINIPVTQNMVPSSRLLVYYIVTGEQTAELVSDSVWLNIEEKCGNQLQVHLSPDADTYSPGQTVSLNMVTGMDSWVALTAVDSAVYGVQRRAKKPLERVFQFLEKSDLGCGAGGGLNNANVFHLAGLTFLTNANADDSQENDEPCKEIIRPRRMLQEKIEEIAAKYKHLVVKKCCYDGVRINHDETCEQRAARISVGPRCVKAFTECCVVASQLRANNSHKDLQLGRLHMKTLLPVSKPEIRSYFPESWLWEVHLVPRRKQLQFALPDSVTTWEIQGVGISNSGICVADTIKAKVFKDVFLEMNIPYSVVRGEQVQLKGTVYNYRTSGMQFCVKMSAVEGICTSESPVIDHQGTKSSKCVRQKVEGSSNHLVTFTVLPLEIGLQNINFSLETSFGKEILVKSLRVVPEGVKRESYSGITLDPRGIYGTISRRKEFPYRIPLDLVPKTEIKRILSVKGLLVGEILSAVLSREGINILTHLPKGSAEAELMSVVPVFYVFHYLETGNHWNIFHSDPLIEKRNLEKKLKEGMVSIMSYRNADYSYSVWKGGSASTWLTAFALRVLGQVHKHVEQNQNSICNSLLWLVENYQLDNGSFKENSQYQPIKLQGTLPVEARENSLYLTAFTVIGIRKAFDICPLVKINTALIKADTFLLENTLPAQSTFTLAISAYALSLGDKTHPQFRSIVSALKREALVKGNPPIYRFWKDSLQHKDSSVPNTGTARMVETTAYALLTSLNLKDINYVNPIIKWLSEEQRYGGGFYSTQDTINAIEGLTEYSLLVKQLRLNMDIDVAYKHKGPLHNYKMTDKNFLGRPVEVLLNDDLVVSTGFGSGLATVHVTTVVHKTSTSEEVCSFYLKIDTQDIEASHYRGYGNSDYKRIVACASYKPSREESSSGSSHAVMDISLPTGINANEEDLKALVEGVDQLFTDYQIKDGHVILQLNSIPSSDFLCVRFRIFELFEVGFLSPATFTVYEYHRPDKQCTMFYSTSNIKIQKVCEGATCKCIEADCGQMQKELDLTISAETRKQTACNPEIAYAYKVIITSITTENVFVKYKATLLDIYKTGEAVAEKDSEITFIKKVTCTNAELVKGRQYLIMGKEALQIKYNFTFRYIYPLDSLTWIEYWPRDTTCSSCQAFLANLDEFAEDIFLNGCEQKLISEEDLGGEQKLISEEDLHHHHHH

SEQ ID NO: 359 - protein, 1676 aa, Artificial Sequence; identical to SEQ ID NO: 355
  hC5 P01031

SEQ ID NO: 360 - protein, 9 aa, Artificial Sequence
  human C5 peptide aa591-599
NMATGMDSW

SEQ ID NO: 361 - protein, 20 aa, Artificial Sequence
  human C5 peptide aa775-794
WEVHLVPRRKQLQFALPDSL

SEQ ID NO: 362 - protein, 121 aa, Artificial Sequence
  HCVR of M1M17628N
EVQLQESGPGLAKPSQTLSLTCSVTGYSITRDYWNWIRKFPGNKLDYMGYISYSGGTYYNPSLKSRFSISRDTSKNQFYLQLNSVTFEDTATYYCARGVSYYGSTYYFDYWGQGTTLTVSS

SEQ ID NO: 363 - protein, 107 aa, Artificial Sequence
  LCVR of M1M17628N
DIQMNQSPSSLSASLGDTITITCHASQNIHVWLNWYQQTPGNIPKLLIYKASNLHTGVPSRFSASGSGTGFTLTISSLQSEDIATYYCQQGQSYPLTFGGGTKLEIK

SEQ ID NO: 364 - protein, 20 aa, Artificial Sequence
  IRBP peptide
GPTHLFQPSLVLDMAKVLLD

SEQ ID NO: 365 - protein, 127 aa, Artificial Sequence
  HCVR of M1M17627N
QVQLQQPGAELVKPGASVKVSCKASGYTFTSYWIHWMRQRPGQGLEWIGRIHPSDSDTNYNQKFKGKATLTVDTSSSTAYMQLSSLTSEDSAVYYCAILPPPPYYYANYGGGTMDYWGRGTSVTVSS

SEQ ID NO: 366 - protein, 107 aa, Artificial Sequence
  LCVR of M1M17627N
DIVMTQSQKFMSTSVGDRVSVTCKASQNVGTNVVWYQQKPGQSPKALIYSASYRYSGVPARFTGSGSGTDFTLTITNVQSEDLAEYICQQYNRSPYTFGGGTKLETK